European Patent Specification EP 3 841 877 B1, published September 6, 2023. Title: GENETICALLY MODIFIED NON-HUMAN ANIMALS EXPRESSING HUMAN EPO. Applicant: Regeneron Pharmaceuticals, Inc. Yale University Institute for Research in Biomedicine (IRB). Application EP. The sequence listing filed with the application follows.

SEQUENCE LISTING (19 sequences)

SEQ ID NO: 1 - DNA, 715 bp, Mus musculus
gatgaagacttgcagcgtggacactggcccagccccgggtcgctaaggagctccggcagctaggcgcggagatgggggtgcccgaacgtcccaccctgctgcttttactctccttgctactgattcctctgggcctcccagtcctctgtgctcccccacgcctcatctgcgacagtcgagttctggagaggtacatcttagaggccaaggaggcagaaaatgtcacgatgggttgtgcagaaggtcccagactgagtgaaaatattacagtcccagataccaaagtcaacttctatgcttggaaaagaatggaggtggaagaacaggccatagaagtttggcaaggcctgtccctgctctcagaagccatcctgcaggcccaggccctgctagccaattcctcccagccaccagagacccttcagcttcatatagacaaagccatcagtggtctacgtagcctcacttcactgcttcgggtactgggagctcagaaggaattgatgtcgcctccagataccaccccacctgctccactccgaacactcacagtggatactttctgcaagctcttccgggtctacgccaacttcctccgggggaaactgaagctgtacacgggagaggtctgcaggagaggggacaggtgacatgctgctgccaccgtggtggaccgacgaacttgctccccgtcactgtgtcatgccaaccctcc

SEQ ID NO: 2 - protein, 192 aa, Mus musculus
MGVPERPTLLLLLSLLLIPLGLPVLCAPPRLICDSRVLERYILEAKEAENVTMGCAEGPRLSENITVPDTKVNFYAWKRMEVEEQAIEVWQGLSLLSEAILQAQALLANSSQPPETLQLHIDKAISGLRSLTSLLRVLGAQKELMSPPDTTPPAPLRTLTVDTFCKLFRVYANFLRGKLKLYTGEVCRRGDR

SEQ ID NO: 3 - DNA, 1340 bp, homo sapiens
cccggagccggaccggggccaccgcgcccgctctgctccgacaccgcgccccctggacagccgccctctcctccaggcccgtggggctggccctgcaccgccgagcttcccgggatgagggcccccggtgtggtcacccggcgcgccccaggtcgctgagggaccccggccaggcgcggagatgggggtgcacgaatgtcctgcctggctgtggcttctcctgtccctgctgtcgctccctctgggcctcccagtcctgggcgccccaccacgcctcatctgtgacagccgagtcctggagaggtacctcttggaggccaaggaggccgagaatatcacgacgggctgtgctgaacactgcagcttgaatgagaatatcactgtcccagacaccaaagttaatttctatgcctggaagaggatggaggtcgggcagcaggccgtagaagtctggcagggcctggccctgctgtcggaagctgtcctgcggggccaggccctgttggtcaactcttcccagccgtgggagcccctgcagctgcatgtggataaagccgtcagtggccttcgcagcctcaccactctgcttcgggctctgggagcccagaaggaagccatctcccctccagatgcggcctcagctgctccactccgaacaatcactgctgacactttccgcaaactcttccgagtctactccaatttcctccggggaaagctgaagctgtacacaggggaggcctgcaggacaggggacagatgaccaggtgtgtccacctgggcatatccaccacctccctcaccaacattgcttgtgccacaccctcccccgccactcctgaaccccgtcgaggggctctcagctcagcgccagcctgtcccatggacactccagtgccagcaatgacatctcaggggccagaggaactgtccagagagcaactctgagatctaaggatgtcacagggccaacttgagggcccagagcaggaagcattcagagagcagctttaaactcagggacagagccatgctgggaagacgcctgagctcactcggcaccctgcaaaatttgatgccaggacacgctttggaggcgatttacctgttttcgcacctaccatcagggacaggatgacctggagaacttaggtggcaagctgtgacttctccaggtctcacgggcatgggcactcccttggtggcaagagcccccttgacaccggggtggtgggaaccatgaagacaggatgggggctggcctctggctctcatggggtccaagttttgtgtattcttcaacctcattgacaagaactgaaaccaccaaaaaaaaaaaa

SEQ ID NO: 4 - protein, 193 aa, homo sapiens
MGVHECPAWLWLLLSLLSLPLGLPVLGAPPRLICDSRVLERYLLEAKEAENITTGCAEHCSLNENITVPDTKVNFYAWKRMEVGQQAVEVWQGLALLSEAVLRGQALLVNSSQPWEPLQLHVDKAVSGLRSLTTLLRALGAQKEAISPPDAASAAPLRTITADTFRKLFRVYSNFLRGKLKLYTGEACRTGDR

SEQ ID NO: 5 - DNA, 226 bp, Artificial Sequence
  synthetic polynucleotide sequence
  misc_feature (1)..(115): mouse sequence
  misc_feature (116)..(128): human Exon 1
  misc_feature (116)..(226): human sequence
tcttccaggctagtggggtgatctggccctacagaacttccaaggatgaagacttgcagcgtggacactggcccagccccgggtcgctaaggagctccggcagctaggcgcggagatgggggtgcacggtgagtactcgcgggctgggcgctcccgcccgcccgggtccctgtttgagcggggatttagcgccccggctattggccaggaggtggctgggttcaag

SEQ ID NO: 6 - DNA, 1054 bp, Artificial sequence
  synthetic polynucleotide sequence
  misc_feature (1)..(115): human Exon 5
  misc_feature (1)..(926): human sequence
  misc_feature (927)..(1054): 5' end of selection cassette
actccgaacaatcactgctgacactttccgcaaactcttccgagtctactccaatttcctccggggaaagctgaagctgtacacaggggaggcctgcaggacaggggacagatgaccaggtgtgtccacctgggcatatccaccacctccctcaccaacattgcttgtgccacaccctcccccgccactcctgaaccccgtcgaggggctctcagctcagcgccagcctgtcccatggacactccagtgccagcaatgacatctcaggggccagaggaactgtccagagagcaactctgagatctaaggatgtcacagggccaacttgagggcccagagcaggaagcattcagagagcagctttaaactcagggacagagccatgctgggaagacgcctgagctcactcggcaccctgcaaaatttgatgccaggacacgctttggaggcgatttacctgttttcgcacctaccatcagggacaggatgacctggagaacttaggtggcaagctgtgacttctccaggtctcacgggcatgggcactcccttggtggcaagagcccccttgacaccggggtggtgggaaccatgaagacaggatgggggctggcctctggctctcatggggtccaagttttgtgtattcttcaacctcattgacaagaactgaaaccaccaatatgactcttggcttttctgttttctgggaacctccaaatcccctggctctgtcccactcctggcagcagtgcagcaggtccaggtccgggaaacgaggggtggagggggctgggccctacgtgctgtctcacacagcctgtctgacctctcgaccctaccgggcctgaggccacaagctctgcctacgctggtcaataaggtgtctccattcaaggcctcaccgcagtaaggcagctgccaacctcgagataacttcgtataatgtatgctatacgaagttatatgcatggcctccgcgccgggttttggcgcctcccgcgggcgcccccctcctcacggcgagcgctgccacgtcagacgaagggcgcag

SEQ ID NO: 7 - DNA, 243 bp, Artificial sequence
  synthetic polynucleotide sequence
  misc_feature (1)..(121): 3' end of selection cassette
  misc_feature (122)..(243): mouse sequence
gcctctgttccacatacacttcattctcagtattgttttgccaagttctaattccatcagacctcgacctgcagcccctagataacttcgtataatgtatgctatacgaagttatgctagcgccaacccgctaggacaagtgctgagtgagctggggccaccgtttgaggaaacaggagccagtacagaggggttcccctttaggggttggtggcaatgggcgaccctggttaatggatcatt

SEQ ID NO: 8 - DNA, 20 bp, Artificial sequence
  synthetic polynucleotide sequence
catctgcgacagtcgagttc

SEQ ID NO: 9 - DNA, 19 bp, Artificial sequence
  synthetic polynucleotide sequence
ccagggagcttaccgtgac

SEQ ID NO: 10 - DNA, 27 bp, Artificial sequence
  synthetic polynucleotide sequence
aggtacatcttagaggccaaggaggca

SEQ ID NO: 11 - DNA, 19 bp, Artificial sequence
  synthetic polynucleotide sequence
acagccgagtcctggagag

SEQ ID NO: 12 - DNA, 19 bp, Artificial sequence
  synthetic polynucleotide sequence
aagccctgagcgtgagttc

SEQ ID NO: 13 - DNA, 26 bp, Artificial sequence
  synthetic polynucleotide sequence
aggccaaggaggccgagaatatcacg

SEQ ID NO: 14 - DNA, 19 bp, Artificial sequence
  synthetic polynucleotide sequence
gagccctgcactggacaac

SEQ ID NO: 15 - DNA, 20 bp, Artificial sequence
  synthetic polynucleotide sequence
tcccatgaacgctgagagtc

SEQ ID NO: 16 - DNA, 28 bp, Artificial sequence
  synthetic polynucleotide sequence
agggtcaaggagccatagacagaatggc

SEQ ID NO: 17 - DNA, 200 bp, Artificial sequence
  synthetic polynucleotide sequence
  misc_feature (1)..(100): mouse sequence
  misc_feature (101)..(200): human sequence
agctctcctaccactagactgctgagacccgctgctctgctcaggactcgatttccagtacacaatctccctctttgaaaagtaccacacatcctggggtgctcttgcatttgtgtgacactttgctagccaggctcagtcctgggttccaggtggggactcaaacacactggcacgagtctacattggatattcttggt

SEQ ID NO: 18 - DNA, 199 bp, Artificial sequence
  synthetic polynucleotide sequence
  misc_feature (1)..(100): 5' end of neomycin cassette
  misc_feature (101)..(199): human sequence
  misc_feature (106)..(139): LoxP
gctccccattcctcactggcccagcccctcttccctactctttctagcccctgcctcatctccctggctgccattgggagcctgccccactggaagccagtcgagataacttcgtataatgtatgctatacgaagttatatgcatggcctccgcgccgggttttggcgcctcccgcgggcgcccccctcctcacggcga

SEQ ID NO: 19 - DNA, 200 bp, Artificial sequence
  synthetic polynucleotide sequence
  misc_feature (1)..(100): 3' neomycin cassette
  misc_feature (101)..(200): mouse Exon 4
cattctcagtattgttttgccaagttctaattccatcagacctcgacctgcagcccctagataacttcgtataatgtatgctatacgaagttatgctagctgtctcatagaggctggcgatctggctcagggacagccagtactgcaaagagtatccttgttcataccttctcctagtggccatctccctgggacagtca